European Patent Specification EP 4 125 996 B1, published August 28, 2024. Title: Ezrin peptide 1 for use in a method of treating COVID-19. Applicant: Dr. Neßelhut Besitzgesellschaft mbH. The sequence listing filed with the application follows.

SEQUENCE LISTING (2 sequences)

SEQ ID NO: 1 - protein, 14 aa, Artificial Sequence
  Tetradecapeptide of human Ezrin
TEKKRRETVEREKE

SEQ ID NO: 2 - protein, 14 aa, Artificial Sequence
  Ezrin derived  polypeptide
GEKKRRETVEREGG